European Patent Application EP 4 570 923 A1, published June 18, 2025. Title: 一种膀胱癌检测试剂盒及检测方法. Applicant: 青岛瑞思德医学检验实验室有限公司. The sequence listing filed with the application follows.

SEQUENCE LISTING (15 sequences)

SEQ ID NO: 1 - DNA, 201 bp, Homo sapiens
  source 1..201: mol_type = genomic DNA
ctgcaggtactttgtgagttttgtcctgcagttccagttccatgaagccctgtgcaaggaggcaggctatgagggcccactgcaccagtgtgacatctaccggtccaccaaggcaggggccaagctccggtgtgtggtgggaagccgggggaagtgggaggcagagaggagcggctggcaaagggtgtggcaggaggtgtc

SEQ ID NO: 2 - DNA, 300 bp, Homo sapiens
  source 1..300: mol_type = genomic DNA
ttcgttttttagtttttttttttcgttttatttttttttttcggggtttaataattcgtttttttaaattatttaaaaacgatttggttcgggcggtcggtttttttattcgttttttagtcgttttttttttttttttttcgtcgttttttttcggcgggcgcggggcgattttttttttcgtcggagcgtgcgggtagcgttttcgaattttagcgtagtttaggaagcggtcggaggagattgttttggtcgcggtggtagttttattcggagtggttgtgatagtagtaatggtaa

SEQ ID NO: 3 - DNA, 321 bp, Homo sapiens
  source 1..321: mol_type = genomic DNA
tttgacaattttgagccaggctttcaggcagcagaggcctgggtggcagtctgtggtgtgaagtggatttagtcacacacagtctgatgttgtaaaccacatgggctctatttaccttcctctcctaggactaggaagattctgtagagtatcggaaagcattggttcatgtgctgccaggattcatgttggctctggtgagccagggacagggaactgacctgcaggcagcccaagcagccacctactcacctcacaatgacagggaccctcatcatacaggtcagggctcaactcaaagacaggcgtggcagtgggaca

SEQ ID NO: 4 - DNA, 15 bp, Homo sapiens
  source 1..15: mol_type = other DNA
tgagttttgtcctgc

SEQ ID NO: 5 - DNA, 19 bp, Homo sapiens
  source 1..19: mol_type = other DNA
acaccggagcttggcccct

SEQ ID NO: 6 - DNA, 18 bp, Homo sapiens
  source 1..18: mol_type = other DNA
aggctatgagggcccact

SEQ ID NO: 7 - DNA, 25 bp, Homo sapiens
  source 1..25: mol_type = other DNA
ttttttttcggcgggcgcggggcga

SEQ ID NO: 8 - DNA, 24 bp, Homo sapiens
  source 1..24: mol_type = other DNA
ccgaataaaactaccaccgcgacc

SEQ ID NO: 9 - DNA, 21 bp, Homo sapiens
  source 1..21: mol_type = other DNA
tcgtcggagcgtgcgggtagc

SEQ ID NO: 10 - DNA, 25 bp, Homo sapiens
  source 1..25: mol_type = other DNA
tttgtagagtatcggaaagtattgg

SEQ ID NO: 11 - DNA, 23 bp, Homo sapiens
  source 1..23: mol_type = other DNA
ctatataataaaaatccctatca

SEQ ID NO: 12 - DNA, 25 bp, Homo sapiens
  source 1..25: mol_type = other DNA
tttgtagagtatcggaaagtattgg

SEQ ID NO: 13 - DNA, 16 bp, Homo sapiens
  source 1..16: mol_type = other DNA
taggatttttatttag

SEQ ID NO: 14 - DNA, 16 bp, Homo sapiens
  source 1..16: mol_type = other DNA
tgtgaatttttgttat

SEQ ID NO: 15 - DNA, 15 bp, Homo sapiens
  source 1..15: mol_type = other DNA
ttttaagggaggagt